European Patent Application EP 4 162 804 A1, published April 12, 2023. Title: MEAT-LIKE FOOD COMPOSITION. Applicant: Spiber Inc. Application EP21822806.2. The sequence listing filed with the application follows.

SEQUENCE LISTING (6 sequences)

SEQ ID NO: 1 - protein, 2375 aa, Artificial Sequence
  PRT799
MHHHHHHSSGSSGPGQQGPYGPGASAAAAAGQNGPGSGQQGPGQSGQYGPGQQGPGQQGPGSSAAAAAGPGQYGPGQQGPSASAAAAAGPGSGQQGPGASGQYGPGQQGPGQQGPGSSAAAAAGQYGSGPGQQGPYGSAAAAAGPGSGQYGQGPYGPGASGPGQYGPGQQGPSASAAAAAGSGQQGPGQYGPYASAAAAAGQYGSGPGQQGPYGPGQSGSGQQGPGQQGPYASAAAAAGPGQQGPYGPGSSAAAAAGQYGYGPGQQGPYGPGASGQNGPGSGQYGPGQQGPGQSAAAAAGPGQQGPYGPGASAAAAAGQYGPGQQGPGQYGPGSSGPGQQGPYGPGSSAAAAAGQYGPGQQGPYGPGQSAAAAAGQYQQGPGQQGPYGPGASGPGQQGPYGPGASAAAAAGPGQYGPGQQGPSASAAAAAGQYGSGPGQYGPYGPGQSGPGSGQQGQGPYGPGASAAAAAGQYGPGQQGPYGPGQSAAAAAGPGSGQYGPGASGQNGPGSGQYGPGQQGPGQSAAAAAGQYQQGPGQQGPYGPGASAAAAAGQYGSGPGQQGPYGPGQSGSGQQGPGQQGPYASAAAAAGPGSGQQGPGASGQQGPYGPGASAAAAAGQNGPGSGQQGPGQSGQYGPGQQGPGQQGPGSSAAAAAGPGQYGPGQQGPSASAAAAAGPGSGQQGPGASGQYGPGQQGPGQQGPGSSAAAAAGQYGSGPGQQGPYGSAAAAAGPGSGQYGQGPYGPGASGPGQYGPGQQGPSASAAAAAGSGQQGPGQYGPYASAAAAAGQYGSGPGQQGPYGPGQSGSGQQGPGQQGPYASAAAAAGPGQQGPYGPGSSAAAAAGQYGYGPGQQGPYGPGASGQNGPGSGQYGPGQQGPGQSAAAAAGPGQQGPYGPGASAAAAAGQYGPGQQGPGQYGPGSSGPGQQGPYGPGSSAAAAAGQYGPGQQGPYGPGQSAAAAAGQYQQGPGQQGPYGPGASGPGQQGPYGPGASAAAAAGPGQYGPGQQGPSASAAAAAGQYGSGPGQYGPYGPGQSGPGSGQQGQGPYGPGASAAAAAGQYGPGQQGPYGPGQSAAAAAGPGSGQYGPGASGQNGPGSGQYGPGQQGPGQSAAAAAGQYQQGPGQQGPYGPGASAAAAAGQYGSGPGQQGPYGPGQSGSGQQGPGQQGPYASAAAAAGPGSGQQGPGASGQQGPYGPGASAAAAAGQNGPGSGQQGPGQSGQYGPGQQGPGQQGPGSSAAAAAGPGQYGPGQQGPSASAAAAAGPGSGQQGPGASGQYGPGQQGPGQQGPGSSAAAAAGQYGSGPGQQGPYGSAAAAAGPGSGQYGQGPYGPGASGPGQYGPGQQGPSASAAAAAGSGQQGPGQYGPYASAAAAAGQYGSGPGQQGPYGPGQSGSGQQGPGQQGPYASAAAAAGPGQQGPYGPGSSAAAAAGQYGYGPGQQGPYGPGASGQNGPGSGQYGPGQQGPGQSAAAAAGPGQQGPYGPGASAAAAAGQYGPGQQGPGQYGPGSSGPGQQGPYGPGSSAAAAAGQYGPGQQGPYGPGQSAAAAAGQYQQGPGQQGPYGPGASGPGQQGPYGPGASAAAAAGPGQYGPGQQGPSASAAAAAGQYGSGPGQYGPYGPGQSGPGSGQQGQGPYGPGASAAAAAGQYGPGQQGPYGPGQSAAAAAGPGSGQYGPGASGQNGPGSGQYGPGQQGPGQSAAAAAGQYQQGPGQQGPYGPGASAAAAAGQYGSGPGQQGPYGPGQSGSGQQGPGQQGPYASAAAAAGPGSGQQGPGASGQQGPYGPGASAAAAAGQNGPGSGQQGPGQSGQYGPGQQGPGQQGPGSSAAAAAGPGQYGPGQQGPSASAAAAAGPGSGQQGPGASGQYGPGQQGPGQQGPGSSAAAAAGQYGSGPGQQGPYGSAAAAAGPGSGQYGQGPYGPGASGPGQYGPGQQGPSASAAAAAGSGQQGPGQYGPYASAAAAAGQYGSGPGQQGPYGPGQSGSGQQGPGQQGPYASAAAAAGPGQQGPYGPGSSAAAAAGQYGYGPGQQGPYGPGASGQNGPGSGQYGPGQQGPGQSAAAAAGPGQQGPYGPGASAAAAAGQYGPGQQGPGQYGPGSSGPGQQGPYGPGSSAAAAAGQYGPGQQGPYGPGQSAAAAAGQYQQGPGQQGPYGPGASGPGQQGPYGPGASAAAAAGPGQYGPGQQGPSASAAAAAGQYGSGPGQYGPYGPGQSGPGSGQQGQGPYGPGASAAAAAGQYGPGQQGPYGPGQSAAAAAGPGSGQYGPGASGQNGPGSGQYGPGQQGPGQSAAAAAGQYQQGPGQQGPYGPGASAAAAAGQYGSGPGQQGPYGPGQSGSGQQGPGQQGPYASAAAAAGPGSGQQGSSVDKLAAALEHHHHHH

SEQ ID NO: 2 - protein, 1190 aa, Artificial Sequence
  PRT966
MHHHHHHSSGSSGPGVFGPYGPGASAAAAAGINGPGSGVFGPGISGIYGPGVFGPGVFGPGSSAAAAAGPGIYGPGVFGPSASAAAAAGPGSGVFGPGASGIYGPGVFGPGVFGPGSSAAAAAGIYGSGPGVFGPYGSAAAAAGPGSGIYGIGPYGPGASGPGIYGPGVFGPSASAAAAAGSGVFGPGIYGPYASAAAAAGIYGSGPGVFGPYGPGISGSGVFGPGVFGPYASAAAAAGPGVFGPYGPGSSAAAAAGIYGYGPGVFGPYGPGASGINGPGSGIYGPGVFGPGISAAAAAGPGVFGPYGPGASAAAAAGIYGPGVFGPGIYGPGSSGPGVFGPYGPGSSAAAAAGIYGPGVFGPYGPGISAAAAAGIYVFGPGVFGPYGPGASGPGVFGPYGPGASAAAAAGPGIYGPGVFGPSASAAAAAGIYGSGPGIYGPYGPGISGPGSGVFGIGPYGPGASAAAAAGIYGPGVFGPYGPGISAAAAAGPGSGIYGPGASGINGPGSGIYGPGVFGPGISAAAAAGIYVFGPGVFGPYGPGASAAAAAGIYGSGPGVFGPYGPGISGSGVFGPGVFGPYASAAAAAGPGSGVFGPGASGPGVFGPYGPGASAAAAAGINGPGSGVFGPGISGIYGPGVFGPGVFGPGSSAAAAAGPGIYGPGVFGPSASAAAAAGPGSGVFGPGASGIYGPGVFGPGVFGPGSSAAAAAGIYGSGPGVFGPYGSAAAAAGPGSGIYGIGPYGPGASGPGIYGPGVFGPSASAAAAAGSGVFGPGIYGPYASAAAAAGIYGSGPGVFGPYGPGISGSGVFGPGVFGPYASAAAAAGPGVFGPYGPGSSAAAAAGIYGYGPGVFGPYGPGASGINGPGSGIYGPGVFGPGISAAAAAGPGVFGPYGPGASAAAAAGIYGPGVFGPGIYGPGSSGPGVFGPYGPGSSAAAAAGIYGPGVFGPYGPGISAAAAAGIYVFGPGVFGPYGPGASGPGVFGPYGPGASAAAAAGPGIYGPGVFGPSASAAAAAGIYGSGPGIYGPYGPGISGPGSGVFGIGPYGPGASAAAAAGIYGPGVFGPYGPGISAAAAAGPGSGIYGPGASGINGPGSGIYGPGVFGPGISAAAAAGIYVFGPGVFGPYGPGASAAAAAGIYGSGPGVFGPYGPGISGSGVFGPGVFGPYASAAAAAGPGSGVFGPGAS

SEQ ID NO: 3 - protein, 601 aa, Artificial Sequence
  PRT918
MHHHHHHSSGSSGPGVFGPYGPGASAAAAAGINGPGSGVFGPGISGIYGPGVFGPGVFGPGSSAAAAAGPGIYGPGVFGPSASAAAAAGPGSGVFGPGASGIYGPGVFGPGVFGPGSSAAAAAGIYGSGPGVFGPYGSAAAAAGPGSGIYGIGPYGPGASGPGIYGPGVFGPSASAAAAAGSGVFGPGIYGPYASAAAAAGIYGSGPGVFGPYGPGISGSGVFGPGVFGPYASAAAAAGPGVFGPYGPGSSAAAAAGIYGYGPGVFGPYGPGASGINGPGSGIYGPGVFGPGISAAAAAGPGVFGPYGPGASAAAAAGIYGPGVFGPGIYGPGSSGPGVFGPYGPGSSAAAAAGIYGPGVFGPYGPGISAAAAAGIYVFGPGVFGPYGPGASGPGVFGPYGPGASAAAAAGPGIYGPGVFGPSASAAAAAGIYGSGPGIYGPYGPGISGPGSGVFGIGPYGPGASAAAAAGIYGPGVFGPYGPGISAAAAAGPGSGIYGPGASGINGPGSGIYGPGVFGPGISAAAAAGIYVFGPGVFGPYGPGASAAAAAGIYGSGPGVFGPYGPGISGSGVFGPGVFGPYASAAAAAGPGSGVFGPGAS

SEQ ID NO: 4 - protein, 608 aa, Artificial Sequence
  PRT313
MHHHHHHSSGSSGPGGQGPYGPGASAAAAAGGNGPGSGQQGPGGSAAAAAGGYGPGGQGPGQQGPGSSAAAAAGPGGYGPGGQGPSASAAAAAGPGSGQQGPGASAAAAAGGYGPGGQGPGQQGPGSSAAAAAGGYGSGPGQQGPYGSAAAAAGPGSGGYGQGPYGPGASAAAAAGPGGYGPGGQGPSASAAAAAGSGQQGPGGYGPYASAAAAAGGYGSGPGQQGPYGPGGSAAAAAGSGQQGPGQQGPYASAAAAAGPGGQGPYGPGSSAAAAAGGYGYGPGGQGPYGPGASAAAAAGGNGPGSGGYGPGQQGPGGSAAAAAGPGGQGPYGPGASAAAAAGGYGPGGQGPGGYGPGSSAAAAAGPGGQGPYGPGSSAAAAAGGYGPGQQGPYGPGGSAAAAAGGYQQGPGGQGPYGPGASAAAAAGPGGQGPYGPGASAAAAAGPGGYGPGGQGPSASAAAAAGGYGSGPGGYGPYGPGGSAAAAAGPGSGQQGQGPYGPGASAAAAAGGYGPGQQGPYGPGGSAAAAAGPGSGGYGPGASAAAAAGGNGPGSGGYGPGQQGPGGSAAAAAGGYQQGPGGQGPYGPGASAAAAAGPGSGQQGPGAS

SEQ ID NO: 5 - protein, 608 aa, Artificial Sequence
  PRT1181
MHHHHHHSSGSSGPGVFGPYGPGASAAAAAGINGPGSGVFGPGISAAAAAGIYGPGVFGPGVFGPGSSAAAAAGPGIYGPGVFGPSASAAAAAGPGSGVFGPGASAAAAAGIYGPGVFGPGVFGPGSSAAAAAGIYGSGPGVFGPYGSAAAAAGPGSGIYGIGPYGPGASAAAAAGPGIYGPGVFGPSASAAAAAGSGVFGPGIYGPYASAAAAAGIYGSGPGVFGPYGPGISAAAAAGSGVFGPGVFGPYASAAAAAGPGVFGPYGPGSSAAAAAGIYGYGPGVFGPYGPGASAAAAAGINGPGSGIYGPGVFGPGISAAAAAGPGVFGPYGPGASAAAAAGIYGPGVFGPGIYGPGSSAAAAAGPGVFGPYGPGSSAAAAAGIYGPGVFGPYGPGISAAAAAGIYVFGPGVFGPYGPGASAAAAAGPGVFGPYGPGASAAAAAGPGIYGPGVFGPSASAAAAAGIYGSGPGIYGPYGPGISAAAAAGPGSGVFGIGPYGPGASAAAAAGIYGPGVFGPYGPGISAAAAAGPGSGIYGPGASAAAAAGINGPGSGIYGPGVFGPGISAAAAAGIYVFGPGVFGPYGPGASAAAAAGPGSGVFGPGAS

SEQ ID NO: 6 - protein, 636 aa, Artificial Sequence
  PRT1010
MHHHHHHSSGSSGPGVFGPYGPGASAAAAAGLINGPGSGVFGPGLISGLIYGPGVFGPGVFGPGSSAAAAAGPGLIYGPGVFGPSASAAAAAGPGSGVFGPGASGLIYGPGVFGPGVFGPGSSAAAAAGLIYGSGPGVFGPYGSAAAAAGPGSGLIYGLIGPYGPGASGPGLIYGPGVFGPSASAAAAAGSGVFGPGLIYGPYASAAAAAGLIYGSGPGVFGPYGPGLISGSGVFGPGVFGPYASAAAAAGPGVFGPYGPGSSAAAAAGLIYGYGPGVFGPYGPGASGLINGPGSGLIYGPGVFGPGLISAAAAAGPGVFGPYGPGASAAAAAGLIYGPGVFGPGLIYGPGSSGPGVFGPYGPGSSAAAAAGLIYGPGVFGPYGPGLISAAAAAGLIYVFGPGVFGPYGPGASGPGVFGPYGPGASAAAAAGPGLIYGPGVFGPSASAAAAAGLIYGSGPGLIYGPYGPGLISGPGSGVFGLIGPYGPGASAAAAAGLIYGPGVFGPYGPGLISAAAAAGPGSGLIYGPGASGLINGPGSGLIYGPGVFGPGLISAAAAAGLIYVFGPGVFGPYGPGASAAAAAGLIYGSGPGVFGPYGPGLISGSGVFGPGVFGPYASAAAAAGPGSGVFGPGAS